European Patent Specification EP 3 710 486 B1, published October 8, 2025. Title: Anti-Factor X antibodies. Applicant: Novo Nordisk A/S. The sequence listing filed with the application follows.

SEQUENCE LISTING (57 sequences)

SEQ ID NO: 1 - protein, 415 aa, Homo sapiens
YNSGKLEEFVQGNLERECMEEKCSFEEAREVFENTERTTEFWKQYVDGDQCESNPCLNGGSCKDDINSYECWCPFGFEGKNCELDVTCNIKNGRCEQFCKNSADNKVVCSCTEGYRLAENQKSCEPAVPFPCGRVSVSQTSKLTRAEAVFPDVDYVNSTEAETILDNITQSTQSFNDFTRVVGGEDAKPGQFPWQVVLNGKVDAFCGGSIVNEKWIVTAAHCVETGVKITVVAGEHNIEETEHTEQKRNVIRIIPHHNYNAAINKYNHDIALLELDEPLVLNSYVTPICIADKEYTNIFLKFGSGYVSGWGRVFHKGRSALVLQYLRVPLVDRATCLRSTKFTIYNNMFCAGFHEGGRDSCQGDSGGPHVTEVEGTSFLTGIISWGEECAMKGKYGIYTKVSRYVNWIKEKTKLT

SEQ ID NO: 2 - protein, 448 aa, Homo sapiens [sequence omitted]

SEQ ID NO: 3 - protein, 2 aa, Artificial Sequence
  Common mimimal epitope
LL

SEQ ID NO: 4 - protein, 117 aa, Homo sapiens
  Antibody heavy chain variable domain
QSVEESGGRLVTPGTPLTLTCTVSGFSLSSYAMSWVRQAPGKGLEWIGIISTSGSTFYATWAKGRFTISKTSTTVDLKIISPTIEDTATYFCARDMWAGSRYDFNIWGPGTLVTVSS

SEQ ID NO: 5 - protein, 113 aa, Artificial Sequence
  Antibody light chain variable domain
ADIVMTQTPASVEAAVGGTVTIKCQASQSISSYLAWYQQKPGQRPKLLIYRASTLESGVPSRFKGSGSGTQFTLTISDLECADAATYYCQTYYYSGGGSYASAFGGGTEVVVK

SEQ ID NO: 6 - protein, 117 aa, Artificial Sequence
  Antibody heavy chain variable domain
EVQLVESGGGQVKPGGSLRLSCAASGFTFSTSSIYWVRQAPGKGLEWVSSISSGSSYIFYADSVKGRFTISRDNAKNSLFLQMNSLRAEDTAVYYCVSGYSRLLDYWGQGTLVTVSS

SEQ ID NO: 7 - protein, 112 aa, Artificial Sequence
  Antibody light chain variable domain
DVVMTQSPLSLPVTLGQPASISCRSSQSLVYSDGNTYLNWFQQRPGQSPRRLIYKVSNRDSGVPDRFSGSGSGTDFTLKISRVEAEDVGFYYCMQGTHWPLTFGGGTKVEIK

SEQ ID NO: 8 - protein, 120 aa, Artificial Sequence
  Single variable domain antibody
EVQLVESGGGVVQPGGSLRLSCAASGRTFSTYAMGWFRQAPGKEREFVAAISWSGSRTYYADSVKGRFTISRDNSKNTVYLQMNSLRPEDTALYYCAADATPANGELDYWGQGTLVTVSS

SEQ ID NO: 9 - protein, 120 aa, Artificial Sequence
  Single variable domain antibody
EVQLVESGGGVVQPGGSLRLSCAASGRTFSTYAMGWFRQAPGKEREFVAAISRRGGRTYYADSVKGRFTISRDNSKNTVYLQMNSLRPEDTALYYCAADATARDGLLDYWGQGTLVTVSS

SEQ ID NO: 10 - protein, 120 aa, Artificial Sequence
  Single variable domain antibody
EVQLVESGGGVVQPGGSLRLSCVASGRTFSRYAMGWFRQAPGKEREFVAAISRRGGSTNYADSVKGRFTISRDNSKNTVYLQMNSLRPEDTALYYCAADYSSGDGYLDYWGQGTLVTVSS

SEQ ID NO: 11 - protein, 120 aa, Artificial Sequence
  Single variable domain antibody
EVQLVESGGGVVQPGGSLRLSCAASGGTLSRYAMGWFRQAPGKEREFVAAITRRGSRTYYADSVKGRFTISRDNSKNTVYLQMNSLRPEDTALYYCAADLAPGDYALDYWGQGTLVTVSS

SEQ ID NO: 12 - protein, 121 aa, Artificial Sequence
  Single variable domain antibody
EVQLVESGGGLVQPGGSLRLSCAASGFTFSNYEMSWVRQAPGKGLEWVSDIGSGGGVSTYYADSVKGRFTISRDNAKNTLYLQMNSLKPEDTAMYYCARGWTYGSDGMDYWGKGTLVTVSS

SEQ ID NO: 13 - protein, 12 aa, Human
SVAQATSSSGEA

SEQ ID NO: 14 - protein, 12 aa, Human
VAQATSSSGEAP

SEQ ID NO: 15 - protein, 12 aa, Human
AQATSSSGEAPD

SEQ ID NO: 16 - protein, 12 aa, Human
QATSSSGEAPDS

SEQ ID NO: 17 - protein, 12 aa, Human
ATSSSGEAPDSI

SEQ ID NO: 18 - protein, 12 aa, Human
TSSSGEAPDSIT

SEQ ID NO: 19 - protein, 12 aa, Human
SSSGEAPDSITW

SEQ ID NO: 20 - protein, 12 aa, Human
SSGEAPDSITWK

SEQ ID NO: 21 - protein, 12 aa, Human
SGEAPDSITWKP

SEQ ID NO: 22 - protein, 12 aa, Human
GEAPDSITWKPY

SEQ ID NO: 23 - protein, 12 aa, Human
EAPDSITWKPYD

SEQ ID NO: 24 - protein, 12 aa, Human
APDSITWKPYDA

SEQ ID NO: 25 - protein, 12 aa, Human
PDSITWKPYDAA

SEQ ID NO: 26 - protein, 12 aa, Human
DSITWKPYDAAD

SEQ ID NO: 27 - protein, 12 aa, Human
SITWKPYDAADL

SEQ ID NO: 28 - protein, 12 aa, Human
ITWKPYDAADLD

SEQ ID NO: 29 - protein, 12 aa, Human
TWKPYDAADLDP

SEQ ID NO: 30 - protein, 12 aa, Human
WKPYDAADLDPT

SEQ ID NO: 31 - protein, 12 aa, Human
KPYDAADLDPTE

SEQ ID NO: 32 - protein, 12 aa, Human
PYDAADLDPTEN

SEQ ID NO: 33 - protein, 12 aa, Human
YDAADLDPTENP

SEQ ID NO: 34 - protein, 12 aa, Human
DAADLDPTENPF

SEQ ID NO: 35 - protein, 12 aa, Human
AADLDPTENPFD

SEQ ID NO: 36 - protein, 12 aa, Human
ADLDPTENPFDL

SEQ ID NO: 37 - protein, 12 aa, Human
DLDPTENPFDLL

SEQ ID NO: 38 - protein, 12 aa, Human
LDPTENPFDLLD

SEQ ID NO: 39 - protein, 12 aa, Human
DPTENPFDLLDF

SEQ ID NO: 40 - protein, 12 aa, Human
PTENPFDLLDFN

SEQ ID NO: 41 - protein, 12 aa, Human
TENPFDLLDFNQ

SEQ ID NO: 42 - protein, 12 aa, Human
ENPFDLLDFNQT

SEQ ID NO: 43 - protein, 12 aa, Human
NPFDLLDFNQTQ

SEQ ID NO: 44 - protein, 12 aa, Human
PFDLLDFNQTQP

SEQ ID NO: 45 - protein, 12 aa, Human
FDLLDFNQTQPE

SEQ ID NO: 46 - protein, 12 aa, Human
DLLDFNQTQPER

SEQ ID NO: 47 - protein, 12 aa, Human
LLDFNQTQPERG

SEQ ID NO: 48 - protein, 12 aa, Human
LDFNQTQPERGD

SEQ ID NO: 49 - protein, 12 aa, Human
DFNQTQPERGDN

SEQ ID NO: 50 - protein, 12 aa, Human
FNQTQPERGDNN

SEQ ID NO: 51 - protein, 12 aa, Human
NQTQPERGDNNL

SEQ ID NO: 52 - protein, 12 aa, Human
QTQPERGDNNLT

SEQ ID NO: 53 - protein, 12 aa, Human
TQPERGDNNLTR

SEQ ID NO: 54 - protein, 120 aa, Artificial
  Single variable domain antibody
EVQLVESGGGVVQPGGSLRLSCAASGRTFSTYSMGWFRQAPGKEREFVAAITRRGSRTYYADSVKGRFTISRDNSKNTVYLQMNSLRPEDTALYYCAADRRPADSYLDYWGQGTLVTVSS

SEQ ID NO: 55 - protein, 121 aa, Artificial sequence
  Single variable domain antibody
EVQLVESGGGVVQPGGSLRLSCAASGFTFSDYAMSWVRQAPGKGLEWVSGITSGGGRTYYADSVKGRFTISRDNSKNTLYLQMNSLRPEDTALYYCAAVRTLGLRGSYDYWGQGTLVTVSS

SEQ ID NO: 56 - protein, 120 aa, Artificial sequence
  Single variable domain antibody
EVQLVESGGGVVQPGGSLRLSCAASGFTFSDYAMSWVRQAPGKGLEWVSGITGGGRTYYADSVKGRFTISRDNSKNTLYLQMNSLRPEDTALYYCAAAILTRTRRTYDYWGQGTLVTVSS

SEQ ID NO: 57 - protein, 121 aa, Artificial sequence
  Single variable domain antibody
EVQLVESGGGVVQPGGSLRLSCVASGFTFSDYAMSWVRQAPGKGLEWVSGITSGSGRTYYADSVKGRFTISRDNSKNTVYLQMNSLRPEDTALYYCAAAILRGYRKTYDYWGQGTLVTVSS